European Patent Specification EP 3 966 337 B1, published June 12, 2024. Title: LIVE IMAGING SYSTEM TO VISUALIZE THE RETRO-TRANSCRIBED VIRAL DNA GENOME. Applicant: INSTITUT PASTEUR. The sequence listing filed with the application follows.

SEQUENCE LISTING (33 sequences)

SEQ ID NO: 1 - DNA, 14 bp, artificial
  consensus
  misc_feature (1)..(6): n is a, t, g or c
  misc_feature (9)..(14): n is a, t, g or c
nnnnnncgnnnnnn

SEQ ID NO: 2 - DNA, 16 bp, artificial
  consensus
  misc_feature (1)..(2): n is a, g, c or t
  misc_feature (4)..(7): n is a, g, c or t
  misc_feature (10)..(13): n is a, g, c or t
  misc_feature (15)..(16): n is a, g, c or t
nntnnnncgnnnnann

SEQ ID NO: 3 - DNA, 16 bp, artificial
  consensus
  misc_feature (1)..(1): n is g, c or t
  misc_feature (4)..(4): n is t or g
  misc_feature (5)..(5): n is a or t
  misc_feature (6)..(6): n is t or c
  misc_feature (7)..(7): n is g or a
  misc_feature (10)..(10): n is t or c
  misc_feature (11)..(11): n is g or a
  misc_feature (12)..(12): n is a or t
  misc_feature (13)..(13): n is a or c
nttnnnncgnnnnaac

SEQ ID NO: 4 - DNA, 16 bp, artificial
  ANCH motif
gtttatgcgcataaac

SEQ ID NO: 5 - DNA, 16 bp, artificial
  ANCH motif
ctttatgcgcataaac

SEQ ID NO: 6 - DNA, 16 bp, artificial
  ANCH motif
gttgtcacgtgacaac

SEQ ID NO: 7 - DNA, 16 bp, artificial
  ANCH motif
tttgtcacgtgacaac

SEQ ID NO: 8 - DNA, 16 bp, artificial
  ANCH motif
cttgtcacgtgacaac

SEQ ID NO: 9 - DNA, 59 bp, artificial
  probe
ggggattgtagggaattccaaattcctgcttttacactcggacctcgtcgacatgcatt

SEQ ID NO: 10 - DNA, 58 bp, artificial
  probe
cttttagctgacatttatcacagctggctattacactcggacctcgtcgacatgcatt

SEQ ID NO: 11 - DNA, 55 bp, artificial
  probe
gtgtgctggtacccatgccagatagacttacactcggacctcgtcgacatgcatt

SEQ ID NO: 12 - DNA, 60 bp, artificial
  probe
aatactggagtattgtatggattttcaggcccttacactcggacctcgtcgacatgcatt

SEQ ID NO: 13 - DNA, 60 bp, artificial
  probe
ttttactggtacagtctcaatagggctaatggttacactcggacctcgtcgacatgcatt

SEQ ID NO: 14 - DNA, 60 bp, artificial
  probe
tatgttgacaggtgtaggtcctactaatactgttacactcggacctcgtcgacatgcatt

SEQ ID NO: 15 - DNA, 54 bp, artificial
  probe
ctaatcctcatcctgtctacttgccattacactcggacctcgtcgacatgcatt

SEQ ID NO: 16 - DNA, 56 bp, artificial
  probe
caatcatcacctgccatctgttttccatttacactcggacctcgtcgacatgcatt

SEQ ID NO: 17 - DNA, 58 bp, artificial
  probe
tttccaaagtggatttctgctgtccctgtattacactcggacctcgtcgacatgcatt

SEQ ID NO: 18 - DNA, 59 bp, artificial
  probe
ttgtggatgaatactgccatttgtactgctgttacactcggacctcgtcgacatgcatt

SEQ ID NO: 19 - DNA, 58 bp, artificial
  probe
ttaagatgttcagcctgatctcttacctgtttacactcggacctcgtcgacatgcatt

SEQ ID NO: 20 - DNA, 56 bp, artificial
  probe
tacagtctacttgtccatgcatggcttcttacactcggacctcgtcgacatgcatt

SEQ ID NO: 21 - DNA, 57 bp, artificial
  probe
tcatgttcatcttgggccttatctattccttacactcggacctcgtcgacatgcatt

SEQ ID NO: 22 - DNA, 60 bp, artificial
  probe
tgtcagttagggtgacaactttttgtcttcctttacactcggacctcgtcgacatgcatt

SEQ ID NO: 23 - DNA, 57 bp, artificial
  probe
tgctcctactatgggttctttctctaactttacactcggacctcgtcgacatgcatt

SEQ ID NO: 24 - DNA, 60 bp, artificial
  probe
tctgttagtgctttggttcctctaaggagtttttacactcggacctcgtcgacatgcatt

SEQ ID NO: 25 - DNA, 59 bp, artificial
  probe
ctgtatgtcattgacagtccagctgtcttttttacactcggacctcgtcgacatgcatt

SEQ ID NO: 26 - DNA, 54 bp, artificial
  probe
tggcagcactataggctgtactgtccttacactcggacctcgtcgacatgcatt

SEQ ID NO: 27 - DNA, 60 bp, artificial
  probe
tctgatgttttttgtctggtgtggtaagtcccttacactcggacctcgtcgacatgcatt

SEQ ID NO: 28 - DNA, 55 bp, artificial
  probe
cctcaacagatgttgtctcagctcctcttacactcggacctcgtcgacatgcatt

SEQ ID NO: 29 - DNA, 54 bp, artificial
  probe
attgctggtgatcctttccatccctgttacactcggacctcgtcgacatgcatt

SEQ ID NO: 30 - DNA, 60 bp, artificial
  probe
tttcttttttaaccctgcgggatgtggtattcttacactcggacctcgtcgacatgcatt

SEQ ID NO: 31 - DNA, 56 bp, artificial
  probe
tttaacttttgggccatccattcctggcttacactcggacctcgtcgacatgcatt

SEQ ID NO: 32 - DNA, 58 bp, artificial
  probe
ccctatctttattgtgacgaggggtcgttgttacactcggacctcgtcgacatgcatt

SEQ ID NO: 33 - protein, 354 aa, Burkholderia cenocepacia
MKPSQFAKGFQARPDITTSEKRTALDRLNAIDGIVKSETPTPAPTKSAKKDIAPPPAPEFTIDPSIDESQQYRAWRLENRYAPGQVIELPLKAIKHSPFNPRHFYLKSSIAELAVNLAKQGQQQAIHVIPDYDNPGTYFVSDGGRRVRALKEANKESVKAIVIDVPIGIQSYKLGYDLNVQRDSQTVFDNAVVWRRFLDDKHFQSQKELSEHLGLDESTVAVALSIGKLPEAIMQEMVARPDRFGSNMAYQVGRYHNARGTEATLRLINKIVSDDLSTRQVSDIVKGRVAAQETPKPAGRQRYAQRLEIKLGGKSVGDLKSYGEDRIELRLRGLPKDKRDAILEQLERMLLSEH